European Patent Specification EP 4 526 683 B1, published December 3, 2025. Title: METHOD FOR IDENTIFYING CANCER PATIENTS THAT BENEFIT FROM ANTI-CLEVER-1 TREATMENT. Applicant: Faron Pharmaceuticals Oy. The sequence listing filed with the application follows.

SEQUENCE LISTING (1 sequence)

SEQ ID NO: 1 - protein, 99 aa, Human
EALASDLPNLGPLRTMHGTPISFSCSRTRAGELMVGEDDARIVQRHLPFEGGLAYGIDQLLEPPGLGARCDHFETRPLRLNTCSICGLEPPCPEGSQEQ